European Patent Application EP 4 603 501 A1, published August 20, 2025. Title: Peptide Having Activity of Promoting Hair Growth and Inhibiting Hair Loss and Uses Thereof. Applicant: CAREGENE CO., LTD. Application KR. The sequence listing filed with the application follows.

SEQUENCE LISTING (17 sequences)

SEQ ID NO: 1 - protein, 6 aa, synthetic construct
HPAAPQ

SEQ ID NO: 2 - DNA, 20 bp, synthetic construct
  source 1..20: mol_type = other DNA
ccagctattgtaacacctca

SEQ ID NO: 3 - DNA, 20 bp, synthetic construct
  source 1..20: mol_type = other DNA
ttcagatgtaggcagctgtc

SEQ ID NO: 4 - DNA, 25 bp, synthetic construct
  source 1..25: mol_type = other DNA
accagcagcgactctgaggaggaac

SEQ ID NO: 5 - DNA, 26 bp, synthetic construct
  source 1..26: mol_type = other DNA
tgaccctcttggcagcaggatagtcc

SEQ ID NO: 6 - DNA, 28 bp, synthetic construct
  source 1..28: mol_type = other DNA
accttcgttgccctctgtgccacagatg

SEQ ID NO: 7 - DNA, 21 bp, synthetic construct
  source 1..21: mol_type = other DNA
aggcccggaggcagtccgggt

SEQ ID NO: 8 - DNA, 20 bp, synthetic construct
  source 1..20: mol_type = other DNA
ggagccaaaagggtcatcat

SEQ ID NO: 9 - DNA, 20 bp, synthetic construct
  source 1..20: mol_type = other DNA
gtgatggcatggactgtggt

SEQ ID NO: 10 - DNA, 20 bp, synthetic construct
  source 1..20: mol_type = other DNA
tgctggtgatgggagttgta

SEQ ID NO: 11 - DNA, 20 bp, synthetic construct
  source 1..20: mol_type = other DNA
cctccaagtagcagccaaag

SEQ ID NO: 12 - DNA, 20 bp, synthetic construct
  source 1..20: mol_type = other DNA
caatgcctctggttcccctt

SEQ ID NO: 13 - DNA, 20 bp, synthetic construct
  source 1..20: mol_type = other DNA
cccctcgaggatttcgacag

SEQ ID NO: 14 - DNA, 22 bp, synthetic construct
  source 1..22: mol_type = other DNA
tctgtcgaacacagtggtacct

SEQ ID NO: 15 - DNA, 23 bp, synthetic construct
  source 1..23: mol_type = other DNA
gtgtgtccatttagctgatgcat

SEQ ID NO: 16 - DNA, 23 bp, synthetic construct
  source 1..23: mol_type = other DNA
atgaactttctgctgtcttgggt

SEQ ID NO: 17 - DNA, 22 bp, synthetic construct
  source 1..22: mol_type = other DNA
tggccttggtgaggtttgatcc